European Patent Application EP 4 793 282 A1, published August 19, 2026. Title: 一种新型微肽MP36及其应用. Applicant: 南京安吉生物科技有限公司. Application CN. The sequence listing filed with the application follows.

SEQUENCE LISTING (5 sequences)

SEQ ID NO: 1 - protein, 36 aa, artificial sequence
MRQGPSTEVPGRAPRPRGPAASRADPSLRPEGGQDP

SEQ ID NO: 2 - DNA, 111 bp, artificial sequence
  source 1..111: mol_type = genomic DNA
atgcggcagggcccctccacggaggtcccagggcgcgctccccggcctcgaggcccggccgccagccgcgcggaccccagcctacgccccgagggaggccaggacccctag

SEQ ID NO: 3 - DNA, 19 bp, artificial sequence
  source 1..19: mol_type = other DNA
agggcccctccacggaggt

SEQ ID NO: 4 - DNA, 19 bp, artificial sequence
  source 1..19: mol_type = other DNA
ctccctcggggcgtaggct

SEQ ID NO: 5 - RNA, 19 nt, artificial sequence
  source 1..19: mol_type = other RNA
ctaaacgaaaccgcttcgt